European Patent Application EP 4 506 452 A1, published February 12, 2025. Title: Transposase with improved biosafety and efficiency. Applicant: Max-Delbrueck-Centrum fuer Molekulare Medizin in der Helmholtz-Gemeinschaft. The sequence listing filed with the application follows.

SEQUENCE LISTING (69 sequences)

SEQ ID NO: 1 - DNA, 1023 bp, synthetic construct
  source 1..1023: mol_type = other DNA
atgggcaaatccaaggagatctcccaggacctgaggaaaagaatcgtggacctgcacaaatctggctcttctctgggcgccatctctaaaagactggccgtgcctaggtccagcgtgcagaccattgtgcggaaatacaaacaccacggaaccacacagccatcttaccgctccggacggcggagagtgctgtcccctagagacgagaggaccctcgtgagaaaagtgcagatcaaccctagaacaaccgccaaagacctggtgaaaatgctggaggagaccggcaccaaggtgtccatctctaccgtgaagcgcgtgctgtaccggcacaacctgaagggacactccgcccggaagaaacctctgctgcagaataggcacaagaaagcccggctgagattcgccaccgcccacggcgataaggatagaaccttttggcgcaacgtgctgtggagcgacgagacaaaaatcgagctgttcgggcacaacgatcaccgctacgtgtggcgcaaaaagggagaggcctgtaagccaaaaaacaccatccccaccgtgaaacacggcggaggctccattatgctgtggggctgctttgccgccggcggaaccggagccctgcacaaaatcgacggcatcatggatgccgtgcagtacgtggacatcctgaaacagcacctgaaaacctctgtgagaaaactgaaactgggccgcaaatgggtgttccagcacgacaatgaccctaagcacacatccaaagtggtggccaaatggctgaaagacaacaaagtgaaagtgctggagtggccttcccagtcccccgatctgaacccaattgagaacctgtgggccgagctgaagaaaagagtgcgggccagacggcctacaaacctgacacagctgcaccagctgtgtcaggaggagtgggccaaaatccaccccaactactgtggcaagctggtggagggatacccaaaacggctgacccaagtgaaacagttcaagggcaacgccaccaagtactga

SEQ ID NO: 2 - DNA, 1122 bp, synthetic construct
  source 1..1122: mol_type = other DNA
atgctggctctgaaactggccggcctggacatcaagttcgagagacagaaactcggcggaggcgcccctgctgttggcggaggacctaaagctgctgacaagggcaaatccaaggagatctcccaggacctgaggaaaagaatcgtggacctgcacaaatctggctcttctctgggcgccatctctaaaagactggccgtgcctaggtccagcgtgcagaccattgtgcggaaatacaaacaccacggaaccacacagccatcttaccgctccggacggcggagagtgctgtcccctagagacgagaggaccctcgtgagaaaagtgcagatcaaccctagaacaaccgccaaagacctggtgaaaatgctggaggagaccggcaccaaggtgtccatctctaccgtgaagcgcgtgctgtaccggcacaacctgaagggacactccgcccggaagaaacctctgctgcagaataggcacaagaaagcccggctgagattcgccaccgcccacggcgataaggatagaaccttttggcgcaacgtgctgtggagcgacgagacaaaaatcgagctgttcgggcacaacgatcaccgctacgtgtggcgcaaaaagggagaggcctgtaagccaaaaaacaccatccccaccgtgaaacacggcggaggctccattatgctgtggggctgctttgccgccggcggaaccggagccctgcacaaaatcgacggcatcatggatgccgtgcagtacgtggacatcctgaaacagcacctgaaaacctctgtgagaaaactgaaactgggccgcaaatgggtgttccagcacgacaatgaccctaagcacacatccaaagtggtggccaaatggctgaaagacaacaaagtgaaagtgctggagtggccttcccagtcccccgatctgaacccaattgagaacctgtgggccgagctgaagaaaagagtgcgggccagacggcctacaaacctgacacagctgcaccagctgtgtcaggaggagtgggccaaaatccaccccaactactgtggcaagctggtggagggatacccaaaacggctgacccaagtgaaacagttcaagggcaacgccaccaagtactga

SEQ ID NO: 3 - RNA, 1297 nt, synthetic construct
  source 1..1297: mol_type = other RNA
acatttgcttctgacacaactgtgttcactagcaacctcaaacagacaccatgggcaaatccaaggagatctcccaggacctgaggaaaagaatcgtggacctgcacaaatctggctcttctctgggcgccatctctaaaagactggccgtgcctaggtccagcgtgcagaccattgtgcggaaatacaaacaccacggaaccacacagccatcttaccgctccggacggcggagagtgctgtcccctagagacgagaggaccctcgtgagaaaagtgcagatcaaccctagaacaaccgccaaagacctggtgaaaatgctggaggagaccggcaccaaggtgtccatctctaccgtgaagcgcgtgctgtaccggcacaacctgaagggacactccgcccggaagaaacctctgctgcagaataggcacaagaaagcccggctgagattcgccaccgcccacggcgataaggatagaaccttttggcgcaacgtgctgtggagcgacgagacaaaaatcgagctgttcgggcacaacgatcaccgctacgtgtggcgcaaaaagggagaggcctgtaagccaaaaaacaccatccccaccgtgaaacacggcggaggctccattatgctgtggggctgctttgccgccggcggaaccggagccctgcacaaaatcgacggcatcatggatgccgtgcagtacgtggacatcctgaaacagcacctgaaaacctctgtgagaaaactgaaactgggccgcaaatgggtgttccagcacgacaatgaccctaagcacacatccaaagtggtggccaaatggctgaaagacaacaaagtgaaagtgctggagtggccttcccagtcccccgatctgaacccaattgagaacctgtgggccgagctgaagaaaagagtgcgggccagacggcctacaaacctgacacagctgcaccagctgtgtcaggaggagtgggccaaaatccaccccaactactgtggcaagctggtggagggatacccaaaacggctgacccaagtgaaacagttcaagggcaacgccaccaagtactgagctcgctttcttgctgtccaatttctattaaaggttcctttgttccctaagtccaactactaaactgggggatattatgaagggccttgagcatctggattctgcctaataaaaaacatttattttcattgcaaaaaaaaaaaaaaaaaaaaaaaaaaaaaaaaaaaaaaaaaaaaaaaaaaaaaaaaaaaaaaaaaaaaaaaaaaaaaaaaaaaaaaaaaaaa

SEQ ID NO: 4 - RNA, 1851 nt, synthetic construct
  source 1..1851: mol_type = other RNA
acatttgcttctgacacaactgtgttcactagcaacctcaaacagacaccatgctggctctgaaactggccggcctggacatcaagttcgagagacagaaactcggcggaggcgcccctgctgttggcggaggacctaaagctgctgacaagggcaaatccaaggagatctcccaggacctgaggaaaagaatcgtggacctgcacaaatctggctcttctctgggcgccatctctaaaagactggccgtgcctaggtccagcgtgcagaccattgtgcggaaatacaaacaccacggaaccacacagccatcttaccgctccggacggcggagagtgctgtcccctagagacgagaggaccctcgtgagaaaagtgcagatcaaccctagaacaaccgccaaagacctggtgaaaatgctggaggagaccggcaccaaggtgtccatctctaccgtgaagcgcgtgctgtaccggcacaacctgaagggacactccgcccggaagaaacctctgctgcagaataggcacaagaaagcccggctgagattcgccaccgcccacggcgataaggatagaaccttttggcgcaacgtgctgtggagcgacgagacaaaaatcgagctgttcgggcacaacgatcaccgctacgtgtggcgcaaaaagggagaggcctgtaagccaaaaaacaccatccccaccgtgaaacacggcggaggctccattatgctgtggggctgctttgccgccggcggaaccggagccctgcacaaaatcgacggcatcatggatgccgtgcagtacgtggacatcctgaaacagcacctgaaaacctctgtgagaaaactgaaactgggccgcaaatgggtgttccagcacgacaatgaccctaagcacacatccaaagtggtggccaaatggctgaaagacaacaaagtgaaagtgctggagtggccttcccagtcccccgatctgaacccaattgagaacctgtgggccgagctgaagaaaagagtgcgggccagacggcctacaaacctgacacagctgcaccagctgtgtcaggaggagtgggccaaaatccaccccaactactgtggcaagctggtggagggatacccaaaacggctgacccaagtgaaacagttcaagggcaacgccaccaagtactgaaatcaacctctggattacaaaatttgtgaaagattgactggtattcttaactatgttgctccttttacgctatgtggatacgctgctttaatgcctttgtatcatgctattgcttcccgtatggctttcattttctcctccttgtataaatcctggttgctgtctctttatgaggagttgtggcccgttgtcaggcaacgtggcgtggtgtgcactgtgtttgctgacgcaacccccactggttggggcattgccaccacctgtcagctcctttccgggactttcgctttccccctccctattgccacggcggaactcatcgccgcctgccttgcccgctgctggacaggggctcggctgttgggcactgacaattccgtggtgttgtcggggaagctgacgtcctttccatggctgctcgcctgtgttgccacctggattctgcgcgggacgtccttctgctacgtcccttcggccctcaatccagcggaccttccttcccgcggcctgctgccggctctgcggcctcttccgcgtcttggccttcgccctcagacgagtcggatctccctttgggccgcctccccgcaaaaaaaaaaaaaaaaaaaaaaaaaaaaaaaaaaaaaaaaaaaaaaaaaaaaaaaaaaaaaaaaaaaaaaaaaaaaaaaaaaaaaaaaaa

SEQ ID NO: 5 - RNA, 1530 nt, synthetic construct
  source 1..1530: mol_type = other RNA
acatttgcttctgacacaactgtgttcactagcaacctcaaacagacaccatgctcgccctcaagctggcggggctggacatcaagttcgagcgccagaagctgggcggcggcgccccggccgtgggcgggggcccgaaggccgccgacaagggcaagtccaaggagatctcgcaggacctccgcaagcggatcgtggacctccacaagtccggcagctccctcggggccatctccaagcgcctggccgtcccgcggtcgtccgtgcagacgatcgtccggaagtacaagcaccacggcaccacgcagccgtcgtacaggtcgggccgccgccgggtgctcagcccccgggacgagcggacgctcgtccggaaggtccagatcaacccgcggaccaccgcgaaggacctcgtcaagatgctcgaggagacgggcaccaaggtgtcgatctccacggtgaagcgggtcctctaccggcacaacctcaaggggcactccgcgcggaagaagcccctgctccagaaccgccacaagaaggcccgcctgcgcttcgccaccgcccacggggacaaggaccggacgttctggcggaacgtcctctggtcggacgagaccaagatcgagctgttcggccacaacgaccaccggtacgtctggcgcaagaagggcgaggcctgcaagcccaagaacaccatccccacggtcaagcacggcgggggctcgatcatgctgtgggggtgcttcgcggccggcgggacgggcgccctccacaagatcgacgggatcatggacgccgtgcagtacgtggacatcctgaagcagcacctcaagacctccgtgcggaagctgaagctcggcaggaagtgggtgttccagcacgacaacgacccgaagcacacgtcgaaggtcgtggcgaagtggctgaaggacaacaaggtgaaggtgctcgagtggccctcccagtcccccgacctgaaccccatcgagaacctgtgggccgagctcaagaagcgggtgcgggcccggaggcccaccaacctcacgcagctgcaccagctctgccaggaggagtgggccaagatccaccccaactactgcggcaagctggtcgagggctacccgaagcggctcacgcaggtcaagcagttcaagggcaacgccacgaaatactgagctcgctttcttgctgtccaatttctattaaaggttcctttgttccctaagtccaactactaaactgggggatattatgaagggccttgagcatctggattctgcctaataaaaaacatttattttcattgcaagctcgctttcttgctgtccaatttctattaaaggttcctttgttccctaagtccaactactaaactgggggatattatgaagggccttgagcatctggattctgcctaataaaaaacatttattttcattgcaaaaaaaaaaaaaaaaaaaaaaaaaaaaaaaaaaaaaaaaaaaaaaaaaaaaaaaaaaaaaaaaaaaaaaaaaaaaaaaaaaaaaaaaaaaa

SEQ ID NO: 6 - RNA, 1396 nt, synthetic construct
  source 1..1396: mol_type = other RNA
acatttgcttctgacacaactgtgttcactagcaacctcaaacagacaccatgctggctctgaaactggccggcctggacatcaagttcgagagacagaaactcggcggaggcgcccctgctgttggcggaggacctaaagctgctgacaagggcaaatccaaggagatctcccaggacctgaggaaaagaatcgtggacctgcacaaatctggctcttctctgggcgccatctctaaaagactggccgtgcctaggtccagcgtgcagaccattgtgcggaaatacaaacaccacggaaccacacagccatcttaccgctccggacggcggagagtgctgtcccctagagacgagaggaccctcgtgagaaaagtgcagatcaaccctagaacaaccgccaaagacctggtgaaaatgctggaggagaccggcaccaaggtgtccatctctaccgtgaagcgcgtgctgtaccggcacaacctgaagggacactccgcccggaagaaacctctgctgcagaataggcacaagaaagcccggctgagattcgccaccgcccacggcgataaggatagaaccttttggcgcaacgtgctgtggagcgacgagacaaaaatcgagctgttcgggcacaacgatcaccgctacgtgtggcgcaaaaagggagaggcctgtaagccaaaaaacaccatccccaccgtgaaacacggcggaggctccattatgctgtggggctgctttgccgccggcggaaccggagccctgcacaaaatcgacggcatcatggatgccgtgcagtacgtggacatcctgaaacagcacctgaaaacctctgtgagaaaactgaaactgggccgcaaatgggtgttccagcacgacaatgaccctaagcacacatccaaagtggtggccaaatggctgaaagacaacaaagtgaaagtgctggagtggccttcccagtcccccgatctgaacccaattgagaacctgtgggccgagctgaagaaaagagtgcgggccagacggcctacaaacctgacacagctgcaccagctgtgtcaggaggagtgggccaaaatccaccccaactactgtggcaagctggtggagggatacccaaaacggctgacccaagtgaaacagttcaagggcaacgccaccaagtactgagctcgctttcttgctgtccaatttctattaaaggttcctttgttccctaagtccaactactaaactgggggatattatgaagggccttgagcatctggattctgcctaataaaaaacatttattttcattgcaaaaaaaaaaaaaaaaaaaaaaaaaaaaaaaaaaaaaaaaaaaaaaaaaaaaaaaaaaaaaaaaaaaaaaaaaaaaaaaaaaaaaaaaaaaa

SEQ ID NO: 7 - RNA, 1372 nt, synthetic construct
  source 1..1372: mol_type = other RNA
acatttgcttctgacacaactgtgttcactagcaacctcaaacagacaccatgctggctctgaaactggccggcctggacatcaagttcgagagacagaaactcggcggaggcgcccctgctgttggcggaggacctaaagctgctgacaagggcaaatccaaggagatctcccaggacctgaggaaaagaatcgtggacctgcacaaatctggctcttctctgggcgccatctctaaaagactggccgtgcctaggtccagcgtgcagaccattgtgcggaaatacaaacaccacggaaccacacagccatcttaccgctccggacggcggagagtgctgtcccctagagacgagaggaccctcgtgagaaaagtgcagatcaaccctagaacaaccgccaaagacctggtgaaaatgctggaggagaccggcaccaaggtgtccatctctaccgtgaagcgcgtgctgtaccggcacaacctgaagggacactccgcccggaagaaacctctgctgcagaataggcacaagaaagcccggctgagattcgccaccgcccacggcgataaggatagaaccttttggcgcaacgtgctgtggagcgacgagacaaaaatcgagctgttcgggcacaacgatcaccgctacgtgtggcgcaaaaagggagaggcctgtaagccaaaaaacaccatccccaccgtgaaacacggcggaggctccattatgctgtggggctgctttgccgccggcggaaccggagccctgcacaaaatcgacggcatcatggatgccgtgcagtacgtggacatcctgaaacagcacctgaaaacctctgtgagaaaactgaaactgggccgcaaatgggtgttccagcacgacaatgaccctaagcacacatccaaagtggtggccaaatggctgaaagacaacaaagtgaaagtgctggagtggccttcccagtcccccgatctgaacccaattgagaacctgtgggccgagctgaagaaaagagtgcgggccagacggcctacaaacctgacacagctgcaccagctgtgtcaggaggagtgggccaaaatccaccccaactactgtggcaagctggtggagggatacccaaaacggctgacccaagtgaaacagttcaagggcaacgccaccaagtactgagctggagcctcggtagccgttcctcctgcccgctgggcctcccaacgggccctcctcccctccttgcaccggcccttcctggtctttgaataaagtctgagtgggcagcaaaaaaaaaaaaaaaaaaaaaaaaaaaaaaaaaaaaaaaaaaaaaaaaaaaaaaaaaaaaaaaaaaaaaaaaaaaaaaaaaaaaaaaaaaa

SEQ ID NO: 8 - RNA, 1506 nt, synthetic construct
  source 1..1506: mol_type = other RNA
acatttgcttctgacacaactgtgttcactagcaacctcaaacagacaccatgctggctctgaaactggccggcctggacatcaagttcgagagacagaaactcggcggaggcgcccctgctgttggcggaggacctaaagctgctgacaagggcaaatccaaggagatctcccaggacctgaggaaaagaatcgtggacctgcacaaatctggctcttctctgggcgccatctctaaaagactggccgtgcctaggtccagcgtgcagaccattgtgcggaaatacaaacaccacggaaccacacagccatcttaccgctccggacggcggagagtgctgtcccctagagacgagaggaccctcgtgagaaaagtgcagatcaaccctagaacaaccgccaaagacctggtgaaaatgctggaggagaccggcaccaaggtgtccatctctaccgtgaagcgcgtgctgtaccggcacaacctgaagggacactccgcccggaagaaacctctgctgcagaataggcacaagaaagcccggctgagattcgccaccgcccacggcgataaggatagaaccttttggcgcaacgtgctgtggagcgacgagacaaaaatcgagctgttcgggcacaacgatcaccgctacgtgtggcgcaaaaagggagaggcctgtaagccaaaaaacaccatccccaccgtgaaacacggcggaggctccattatgctgtggggctgctttgccgccggcggaaccggagccctgcacaaaatcgacggcatcatggatgccgtgcagtacgtggacatcctgaaacagcacctgaaaacctctgtgagaaaactgaaactgggccgcaaatgggtgttccagcacgacaatgaccctaagcacacatccaaagtggtggccaaatggctgaaagacaacaaagtgaaagtgctggagtggccttcccagtcccccgatctgaacccaattgagaacctgtgggccgagctgaagaaaagagtgcgggccagacggcctacaaacctgacacagctgcaccagctgtgtcaggaggagtgggccaaaatccaccccaactactgtggcaagctggtggagggatacccaaaacggctgacccaagtgaaacagttcaagggcaacgccaccaagtactgagctcgctttcttgctgtccaatttctattaaaggttcctttgttccctaagtccaactactaaactgggggatattatgaagggccttgagcatctggattctgcctaataaaaaacatttattttcattgcaagctggagcctcggtagccgttcctcctgcccgctgggcctcccaacgggccctcctcccctccttgcaccggcccttcctggtctttgaataaagtctgagtgggcagcaaaaaaaaaaaaaaaaaaaaaaaaaaaaaaaaaaaaaaaaaaaaaaaaaaaaaaaaaaaaaaaaaaaaaaaaaaaaaaaaaaaaaaaaaaa

SEQ ID NO: 9 - RNA, 1369 nt, synthetic construct
  source 1..1369: mol_type = other RNA
acatttgcttctgacacaactgtgttcactagcaacctcaaacagacaccatgctggctctgaaactggccggcctggacatcaagttcgagagacagaaactcggcggaggcgcccctgctgttggcggaggacctaaagctgctgacaagggcaaatccaaggagatctcccaggacctgaggaaaagaatcgtggacctgcacaaatctggctcttctctgggcgccatctctaaaagactggccgtgcctaggtccagcgtgcagaccattgtgcggaaatacaaacaccacggaaccacacagccatcttaccgctccggacggcggagagtgctgtcccctagagacgagaggaccctcgtgagaaaagtgcagatcaaccctagaacaaccgccaaagacctggtgaaaatgctggaggagaccggcaccaaggtgtccatctctaccgtgaagcgcgtgctgtaccggcacaacctgaagggacactccgcccggaagaaacctctgctgcagaataggcacaagaaagcccggctgagattcgccaccgcccacggcgataaggatagaaccttttggcgcaacgtgctgtggagcgacgagacaaaaatcgagctgttcgggcacaacgatcaccgctacgtgtggcgcaaaaagggagaggcctgtaagccaaaaaacaccatccccaccgtgaaacacggcggaggctccattatgctgtggggctgctttgccgccggcggaaccggagccctgcacaaaatcgacggcatcatggatgccgtgcagtacgtggacatcctgaaacagcacctgaaaacctctgtgagaaaactgaaactgggccgcaaatgggtgttccagcacgacaatgaccctaagcacacatccaaagtggtggccaaatggctgaaagacaacaaagtgaaagtgctggagtggccttcccagtcccccgatctgaacccaattgagaacctgtgggccgagctgaagaaaagagtgcgggccagacggcctacaaacctgacacagctgcaccagctgtgtcaggaggagtgggccaaaatccaccccaactactgtggcaagctggtggagggatacccaaaacggctgacccaagtgaaacagttcaagggcaacgccaccaagtactgagctcgctttcttgctgtccaatttctattaaaggttcctttgttccctaagtccaactactaaactgggggatattatgaagggccttgagcatctggattctgcctaaaaaaaaaaaaaaaaaaaaaaaaaaaaaaaaaaaaaaaaaaaaaaaaaaaaaaaaaaaaaaaaaaaaaaaaaaaaaaaaaaaaaaaaaa

SEQ ID NO: 10 - RNA, 1525 nt, synthetic construct
  source 1..1525: mol_type = other RNA
actcactatttgttttcgcgcccagttgcaaaaagtgtcgccaccatgctggctctgaaactggccggcctggacatcaagttcgagagacagaaactcggcggaggcgcccctgctgttggcggaggacctaaagctgctgacaagggcaaatccaaggagatctcccaggacctgaggaaaagaatcgtggacctgcacaaatctggctcttctctgggcgccatctctaaaagactggccgtgcctaggtccagcgtgcagaccattgtgcggaaatacaaacaccacggaaccacacagccatcttaccgctccggacggcggagagtgctgtcccctagagacgagaggaccctcgtgagaaaagtgcagatcaaccctagaacaaccgccaaagacctggtgaaaatgctggaggagaccggcaccaaggtgtccatctctaccgtgaagcgcgtgctgtaccggcacaacctgaagggacactccgcccggaagaaacctctgctgcagaataggcacaagaaagcccggctgagattcgccaccgcccacggcgataaggatagaaccttttggcgcaacgtgctgtggagcgacgagacaaaaatcgagctgttcgggcacaacgatcaccgctacgtgtggcgcaaaaagggagaggcctgtaagccaaaaaacaccatccccaccgtgaaacacggcggaggctccattatgctgtggggctgctttgccgccggcggaaccggagccctgcacaaaatcgacggcatcatggatgccgtgcagtacgtggacatcctgaaacagcacctgaaaacctctgtgagaaaactgaaactgggccgcaaatgggtgttccagcacgacaatgaccctaagcacacatccaaagtggtggccaaatggctgaaagacaacaaagtgaaagtgctggagtggccttcccagtcccccgatctgaacccaattgagaacctgtgggccgagctgaagaaaagagtgcgggccagacggcctacaaacctgacacagctgcaccagctgtgtcaggaggagtgggccaaaatccaccccaactactgtggcaagctggtggagggatacccaaaacggctgacccaagtgaaacagttcaagggcaacgccaccaagtactgagctcgctttcttgctgtccaatttctattaaaggttcctttgttccctaagtccaactactaaactgggggatattatgaagggccttgagcatctggattctgcctaataaaaaacatttattttcattgcaagctcgctttcttgctgtccaatttctattaaaggttcctttgttccctaagtccaactactaaactgggggatattatgaagggccttgagcatctggattctgcctaataaaaaacatttattttcattgcaaaaaaaaaaaaaaaaaaaaaaaaaaaaaaaaaaaaaaaaaaaaaaaaaaaaaaaaaaaaaaaaaaaaaaaaaaaaaaaaaaaaaaaaaaaa

SEQ ID NO: 11 - RNA, 1525 nt, synthetic construct
  source 1..1525: mol_type = other RNA
actcactatttgttttcgcgcccagttgcaaaaagtgtcgccaccatgctagcactaaaactcgcgggactcgatatcaagttcgaaagacagaagctgggcggcggcgccccggccgtgggcgggggcccgaaggccgccgacaagggcaagtccaaggagatctcgcaggacctccgcaagcggatcgtggacctccacaagtccggcagctccctcggggccatctccaagcgcctggccgtcccgcggtcgtccgtgcagacgatcgtccggaagtacaagcaccacggcaccacgcagccgtcgtacaggtcgggccgccgccgggtgctcagcccccgggacgagcggacgctcgtccggaaggtccagatcaacccgcggaccaccgcgaaggacctcgtcaagatgctcgaggagacgggcaccaaggtgtcgatctccacggtgaagcgggtcctctaccggcacaacctcaaggggcactccgcgcggaagaagcccctgctccagaaccgccacaagaaggcccgcctgcgcttcgccaccgcccacggggacaaggaccggacgttctggcggaacgtcctctggtcggacgagaccaagatcgagctgttcggccacaacgaccaccggtacgtctggcgcaagaagggcgaggcctgcaagcccaagaacaccatccccacggtcaagcacggcgggggctcgatcatgctgtgggggtgcttcgcggccggcgggacgggcgccctccacaagatcgacgggatcatggacgccgtgcagtacgtggacatcctgaagcagcacctcaagacctccgtgcggaagctgaagctcggcaggaagtgggtgttccagcacgacaacgacccgaagcacacgtcgaaggtcgtggcgaagtggctgaaggacaacaaggtgaaggtgctcgagtggccctcccagtcccccgacctgaaccccatcgagaacctgtgggccgagctcaagaagcgggtgcgggcccggaggcccaccaacctcacgcagctgcaccagctctgccaggaggagtgggccaagatccaccccaactactgcggcaagctggtcgagggctacccgaagcggctcacgcaggtcaagcagttcaagggcaacgccacgaaatactgagctcgctttcttgctgtccaatttctattaaaggttcctttgttccctaagtccaactactaaactgggggatattatgaagggccttgagcatctggattctgcctaataaaaaacatttattttcattgcaagctcgctttcttgctgtccaatttctattaaaggttcctttgttccctaagtccaactactaaactgggggatattatgaagggccttgagcatctggattctgcctaataaaaaacatttattttcattgcaaaaaaaaaaaaaaaaaaaaaaaaaaaaaaaaaaaaaaaaaaaaaaaaaaaaaaaaaaaaaaaaaaaaaaaaaaaaaaaaaaaaaaaaaaaa

SEQ ID NO: 12 - RNA, 1957 nt, synthetic construct
  source 1..1957: mol_type = other RNA
gaggaattcggggctgaaggatgcccagaaggtaccccattgtatgggatctgatctggggcctcggtgcacatgctttacatgtgtttagtcgaggttaaaaaaacgtctaggccccccgaaccacggggacgtggttttccatggaccgccaccatgctcgccctcaagctggcggggctggacatcaagttcgagcgccagaagctgggcggcggcgccccggccgtgggcgggggcccgaaggccgccgacaagggcaagtccaaggagatctcgcaggacctccgcaagcggatcgtggacctccacaagtccggcagctccctcggggccatctccaagcgcctggccgtcccgcggtcgtccgtgcagacgatcgtccggaagtacaagcaccacggcaccacgcagccgtcgtacaggtcgggccgccgccgggtgctcagcccccgggacgagcggacgctcgtccggaaggtccagatcaacccgcggaccaccgcgaaggacctcgtcaagatgctcgaggagacgggcaccaaggtgtcgatctccacggtgaagcgggtcctctaccggcacaacctcaaggggcactccgcgcggaagaagcccctgctccagaaccgccacaagaaggcccgcctgcgcttcgccaccgcccacggggacaaggaccggacgttctggcggaacgtcctctggtcggacgagaccaagatcgagctgttcggccacaacgaccaccggtacgtctggcgcaagaagggcgaggcctgcaagcccaagaacaccatccccacggtcaagcacggcgggggctcgatcatgctgtgggggtgcttcgcggccggcgggacgggcgccctccacaagatcgacgggatcatggacgccgtgcagtacgtggacatcctgaagcagcacctcaagacctccgtgcggaagctgaagctcggcaggaagtgggtgttccagcacgacaacgacccgaagcacacgtcgaaggtcgtggcgaagtggctgaaggacaacaaggtgaaggtgctcgagtggccctcccagtcccccgacctgaaccccatcgagaacctgtgggccgagctcaagaagcgggtgcgggcccggaggcccaccaacctcacgcagctgcaccagctctgccaggaggagtgggccaagatccaccccaactactgcggcaagctggtcgagggctacccgaagcggctcacgcaggtcaagcagttcaagggcaacgccacgaaatactgaaatcaacctctggattacaaaatttgtgaaagattgactggtattcttaactatgttgctccttttacgctatgtggatacgctgctttaatgcctttgtatcatgctattgcttcccgtatggctttcattttctcctccttgtataaatcctggttgctgtctctttatgaggagttgtggcccgttgtcaggcaacgtggcgtggtgtgcactgtgtttgctgacgcaacccccactggttggggcattgccaccacctgtcagctcctttccgggactttcgctttccccctccctattgccacggcggaactcatcgccgcctgccttgcccgctgctggacaggggctcggctgttgggcactgacaattccgtggtgttgtcggggaagctgacgtcctttccatggctgctcgcctgtgttgccacctggattctgcgcgggacgtccttctgctacgtcccttcggccctcaatccagcggaccttccttcccgcggcctgctgccggctctgcggcctcttccgcgtcttggccttcgccctcagacgagtcggatctccctttgggccgcctccccgcaaaaaaaaaaaaaaaaaaaaaaaaaaaaaaaaaaaaaaaaaaaaaaaaaaaaaaaaaaaaaaaaaaaaaaaaaaaaaaaaaaaaaaaaaa

SEQ ID NO: 13 - RNA, 1868 nt, synthetic construct
  source 1..1868: mol_type = other RNA
ataattcaaaatcaatcagcatcacaacatcaagcatcaatcatcaacacatcaaagagacaccaccatgctggctctgaaactggccggcctggacatcaagttcgagagacagaaactcggcggaggcgcccctgctgttggcggaggacctaaagctgctgacaagggcaaatccaaggagatctcccaggacctgaggaaaagaatcgtggacctgcacaaatctggctcttctctgggcgccatctctaaaagactggccgtgcctaggtccagcgtgcagaccattgtgcggaaatacaaacaccacggaaccacacagccatcttaccgctccggacggcggagagtgctgtcccctagagacgagaggaccctcgtgagaaaagtgcagatcaaccctagaacaaccgccaaagacctggtgaaaatgctggaggagaccggcaccaaggtgtccatctctaccgtgaagcgcgtgctgtaccggcacaacctgaagggacactccgcccggaagaaacctctgctgcagaataggcacaagaaagcccggctgagattcgccaccgcccacggcgataaggatagaaccttttggcgcaacgtgctgtggagcgacgagacaaaaatcgagctgttcgggcacaacgatcaccgctacgtgtggcgcaaaaagggagaggcctgtaagccaaaaaacaccatccccaccgtgaaacacggcggaggctccattatgctgtggggctgctttgccgccggcggaaccggagccctgcacaaaatcgacggcatcatggatgccgtgcagtacgtggacatcctgaaacagcacctgaaaacctctgtgagaaaactgaaactgggccgcaaatgggtgttccagcacgacaatgaccctaagcacacatccaaagtggtggccaaatggctgaaagacaacaaagtgaaagtgctggagtggccttcccagtcccccgatctgaacccaattgagaacctgtgggccgagctgaagaaaagagtgcgggccagacggcctacaaacctgacacagctgcaccagctgtgtcaggaggagtgggccaaaatccaccccaactactgtggcaagctggtggagggatacccaaaacggctgacccaagtgaaacagttcaagggcaacgccaccaagtactgaaatcaacctctggattacaaaatttgtgaaagattgactggtattcttaactatgttgctccttttacgctatgtggatacgctgctttaatgcctttgtatcatgctattgcttcccgtatggctttcattttctcctccttgtataaatcctggttgctgtctctttatgaggagttgtggcccgttgtcaggcaacgtggcgtggtgtgcactgtgtttgctgacgcaacccccactggttggggcattgccaccacctgtcagctcctttccgggactttcgctttccccctccctattgccacggcggaactcatcgccgcctgccttgcccgctgctggacaggggctcggctgttgggcactgacaattccgtggtgttgtcggggaagctgacgtcctttccatggctgctcgcctgtgttgccacctggattctgcgcgggacgtccttctgctacgtcccttcggccctcaatccagcggaccttccttcccgcggcctgctgccggctctgcggcctcttccgcgtcttggccttcgccctcagacgagtcggatctccctttgggccgcctccccgcaaaaaaaaaaaaaaaaaaaaaaaaaaaaaaaaaaaaaaaaaaaaaaaaaaaaaaaaaaaaaaaaaaaaaaaaaaaaaaaaaaaaaaaaaa

SEQ ID NO: 14 - RNA, 1868 nt, synthetic construct
  source 1..1868: mol_type = other RNA
ataattcaaaatcaatcagcatcacaacatcaagcatcaatcatcaacacatcaaagagacaccaccatgctagcactaaaactcgcgggactcgatatcaagttcgaaagacagaagctgggcggcggcgccccggccgtgggcgggggcccgaaggccgccgacaagggcaagtccaaggagatctcgcaggacctccgcaagcggatcgtggacctccacaagtccggcagctccctcggggccatctccaagcgcctggccgtcccgcggtcgtccgtgcagacgatcgtccggaagtacaagcaccacggcaccacgcagccgtcgtacaggtcgggccgccgccgggtgctcagcccccgggacgagcggacgctcgtccggaaggtccagatcaacccgcggaccaccgcgaaggacctcgtcaagatgctcgaggagacgggcaccaaggtgtcgatctccacggtgaagcgggtcctctaccggcacaacctcaaggggcactccgcgcggaagaagcccctgctccagaaccgccacaagaaggcccgcctgcgcttcgccaccgcccacggggacaaggaccggacgttctggcggaacgtcctctggtcggacgagaccaagatcgagctgttcggccacaacgaccaccggtacgtctggcgcaagaagggcgaggcctgcaagcccaagaacaccatccccacggtcaagcacggcgggggctcgatcatgctgtgggggtgcttcgcggccggcgggacgggcgccctccacaagatcgacgggatcatggacgccgtgcagtacgtggacatcctgaagcagcacctcaagacctccgtgcggaagctgaagctcggcaggaagtgggtgttccagcacgacaacgacccgaagcacacgtcgaaggtcgtggcgaagtggctgaaggacaacaaggtgaaggtgctcgagtggccctcccagtcccccgacctgaaccccatcgagaacctgtgggccgagctcaagaagcgggtgcgggcccggaggcccaccaacctcacgcagctgcaccagctctgccaggaggagtgggccaagatccaccccaactactgcggcaagctggtcgagggctacccgaagcggctcacgcaggtcaagcagttcaagggcaacgccacgaaatactgaaatcaacctctggattacaaaatttgtgaaagattgactggtattcttaactatgttgctccttttacgctatgtggatacgctgctttaatgcctttgtatcatgctattgcttcccgtatggctttcattttctcctccttgtataaatcctggttgctgtctctttatgaggagttgtggcccgttgtcaggcaacgtggcgtggtgtgcactgtgtttgctgacgcaacccccactggttggggcattgccaccacctgtcagctcctttccgggactttcgctttccccctccctattgccacggcggaactcatcgccgcctgccttgcccgctgctggacaggggctcggctgttgggcactgacaattccgtggtgttgtcggggaagctgacgtcctttccatggctgctcgcctgtgttgccacctggattctgcgcgggacgtccttctgctacgtcccttcggccctcaatccagcggaccttccttcccgcggcctgctgccggctctgcggcctcttccgcgtcttggccttcgccctcagacgagtcggatctccctttgggccgcctccccgcaaaaaaaaaaaaaaaaaaaaaaaaaaaaaaaaaaaaaaaaaaaaaaaaaaaaaaaaaaaaaaaaaaaaaaaaaaaaaaaaaaaaaaaaaa

SEQ ID NO: 15-21 - skipped (7 entries)

SEQ ID NO: 22 - RNA, 1530 nt, synthetic construct
  source 1..1530: mol_type = other RNA
acatttgcttctgacacaactgtgttcactagcaacctcaaacagacaccatgctcgctcttaagctggcgggactggacatcgtcaagaaggaccaaaagctgggcggaggtgccccagctgttggaggtggcccgaaggctgccgacaagggtaagtccaaggagatctcgcaggacctccgcaagcggatcgtggacctccacaagtccggcagctccctcggggccatctccaagcgcctggccgtcccgcggtcgtccgtgcagacgatcgtccggaagtacaagcaccacggcaccacgcagccgtcgtacaggtcgggccgccgccgggtgctcagcccccgggacgagcggacgctcgtccggaaggtccagatcaacccgcggaccaccgcgaaggacctcgtcaagatgctcgaggagacgggcaccaaggtgtcgatctccacggtgaagcgggtcctctaccggcacaacctcaaggggcactccgcgcggaagaagcccctgctccagaaccgccacaagaaggcccgcctgcgcttcgccaccgcccacggggacaaggaccggacgttctggcggaacgtcctctggtcggacgagaccaagatcgagctgttcggccacaacgaccaccggtacgtctggcgcaagaagggcgaggcctgcaagcccaagaacaccatccccacggtcaagcacggcgggggctcgatcatgctgtgggggtgcttcgcggccggcgggacgggcgccctccacaagatcgacgggatcatggacgccgtgcagtacgtggacatcctgaagcagcacctcaagacctccgtgcggaagctgaagctcggcaggaagtgggtgttccagcacgacaacgacccgaagcacacgtcgaaggtcgtggcgaagtggctgaaggacaacaaggtgaaggtgctcgagtggccctcccagtcccccgacctgaaccccatcgagaacctgtgggccgagctcaagaagcgggtgcgggcccggaggcccaccaacctcacgcagctgcaccagctctgccaggaggagtgggccaagatccaccccaactactgcggcaagctggtcgagggctacccgaagcggctcacgcaggtcaagcagttcaagggcaacgccacgaaatactgagctcgctttcttgctgtccaatttctattaaaggttcctttgttccctaagtccaactactaaactgggggatattatgaagggccttgagcatctggattctgcctaataaaaaacatttattttcattgcaagctcgctttcttgctgtccaatttctattaaaggttcctttgttccctaagtccaactactaaactgggggatattatgaagggccttgagcatctggattctgcctaataaaaaacatttattttcattgcaaaaaaaaaaaaaaaaaaaaaaaaaaaaaaaaaaaaaaaaaaaaaaaaaaaaaaaaaaaaaaaaaaaaaaaaaaaaaaaaaaaaaaaaaaaa

SEQ ID NO: 23 - RNA, 1530 nt, synthetic construct
  source 1..1530: mol_type = other RNA
acatttgcttctgacacaactgtgttcactagcaacctcaaacagacaccatgctcgctcttaagctggcgggactggacatcaagttcttcgagcaaaagctgggcggaggtgccccagctgttggaggtggcccgaaggctgccgacaagggtaagtccaaggagatctcgcaggacctccgcaagcggatcgtggacctccacaagtccggcagctccctcggggccatctccaagcgcctggccgtcccgcggtcgtccgtgcagacgatcgtccggaagtacaagcaccacggcaccacgcagccgtcgtacaggtcgggccgccgccgggtgctcagcccccgggacgagcggacgctcgtccggaaggtccagatcaacccgcggaccaccgcgaaggacctcgtcaagatgctcgaggagacgggcaccaaggtgtcgatctccacggtgaagcgggtcctctaccggcacaacctcaaggggcactccgcgcggaagaagcccctgctccagaaccgccacaagaaggcccgcctgcgcttcgccaccgcccacggggacaaggaccggacgttctggcggaacgtcctctggtcggacgagaccaagatcgagctgttcggccacaacgaccaccggtacgtctggcgcaagaagggcgaggcctgcaagcccaagaacaccatccccacggtcaagcacggcgggggctcgatcatgctgtgggggtgcttcgcggccggcgggacgggcgccctccacaagatcgacgggatcatggacgccgtgcagtacgtggacatcctgaagcagcacctcaagacctccgtgcggaagctgaagctcggcaggaagtgggtgttccagcacgacaacgacccgaagcacacgtcgaaggtcgtggcgaagtggctgaaggacaacaaggtgaaggtgctcgagtggccctcccagtcccccgacctgaaccccatcgagaacctgtgggccgagctcaagaagcgggtgcgggcccggaggcccaccaacctcacgcagctgcaccagctctgccaggaggagtgggccaagatccaccccaactactgcggcaagctggtcgagggctacccgaagcggctcacgcaggtcaagcagttcaagggcaacgccacgaaatactgagctcgctttcttgctgtccaatttctattaaaggttcctttgttccctaagtccaactactaaactgggggatattatgaagggccttgagcatctggattctgcctaataaaaaacatttattttcattgcaagctcgctttcttgctgtccaatttctattaaaggttcctttgttccctaagtccaactactaaactgggggatattatgaagggccttgagcatctggattctgcctaataaaaaacatttattttcattgcaaaaaaaaaaaaaaaaaaaaaaaaaaaaaaaaaaaaaaaaaaaaaaaaaaaaaaaaaaaaaaaaaaaaaaaaaaaaaaaaaaaaaaaaaaaa

SEQ ID NO: 24 - RNA, 1530 nt, synthetic construct
  source 1..1530: mol_type = other RNA
acatttgcttctgacacaactgtgttcactagcaacctcaaacagacaccatgctcgctcttaagctggcgggactggacatcaagatccgagagatcaagctgggcggaggtgccccagctgttggaggtggcccgaaggctgccgacaagggtaagtccaaggagatctcgcaggacctccgcaagcggatcgtggacctccacaagtccggcagctccctcggggccatctccaagcgcctggccgtcccgcggtcgtccgtgcagacgatcgtccggaagtacaagcaccacggcaccacgcagccgtcgtacaggtcgggccgccgccgggtgctcagcccccgggacgagcggacgctcgtccggaaggtccagatcaacccgcggaccaccgcgaaggacctcgtcaagatgctcgaggagacgggcaccaaggtgtcgatctccacggtgaagcgggtcctctaccggcacaacctcaaggggcactccgcgcggaagaagcccctgctccagaaccgccacaagaaggcccgcctgcgcttcgccaccgcccacggggacaaggaccggacgttctggcggaacgtcctctggtcggacgagaccaagatcgagctgttcggccacaacgaccaccggtacgtctggcgcaagaagggcgaggcctgcaagcccaagaacaccatccccacggtcaagcacggcgggggctcgatcatgctgtgggggtgcttcgcggccggcgggacgggcgccctccacaagatcgacgggatcatggacgccgtgcagtacgtggacatcctgaagcagcacctcaagacctccgtgcggaagctgaagctcggcaggaagtgggtgttccagcacgacaacgacccgaagcacacgtcgaaggtcgtggcgaagtggctgaaggacaacaaggtgaaggtgctcgagtggccctcccagtcccccgacctgaaccccatcgagaacctgtgggccgagctcaagaagcgggtgcgggcccggaggcccaccaacctcacgcagctgcaccagctctgccaggaggagtgggccaagatccaccccaactactgcggcaagctggtcgagggctacccgaagcggctcacgcaggtcaagcagttcaagggcaacgccacgaaatactgagctcgctttcttgctgtccaatttctattaaaggttcctttgttccctaagtccaactactaaactgggggatattatgaagggccttgagcatctggattctgcctaataaaaaacatttattttcattgcaagctcgctttcttgctgtccaatttctattaaaggttcctttgttccctaagtccaactactaaactgggggatattatgaagggccttgagcatctggattctgcctaataaaaaacatttattttcattgcaaaaaaaaaaaaaaaaaaaaaaaaaaaaaaaaaaaaaaaaaaaaaaaaaaaaaaaaaaaaaaaaaaaaaaaaaaaaaaaaaaaaaaaaaaaa

SEQ ID NO: 25 - RNA, 1530 nt, synthetic construct
  source 1..1530: mol_type = other RNA
acatttgcttctgacacaactgtgttcactagcaacctcaaacagacaccatgctcgctcttaagctggcgggactggacatccaagtcgagctccgaaagctgggcggaggtgccccagctgttggaggtggcccgaaggctgccgacaagggtaagtccaaggagatctcgcaggacctccgcaagcggatcgtggacctccacaagtccggcagctccctcggggccatctccaagcgcctggccgtcccgcggtcgtccgtgcagacgatcgtccggaagtacaagcaccacggcaccacgcagccgtcgtacaggtcgggccgccgccgggtgctcagcccccgggacgagcggacgctcgtccggaaggtccagatcaacccgcggaccaccgcgaaggacctcgtcaagatgctcgaggagacgggcaccaaggtgtcgatctccacggtgaagcgggtcctctaccggcacaacctcaaggggcactccgcgcggaagaagcccctgctccagaaccgccacaagaaggcccgcctgcgcttcgccaccgcccacggggacaaggaccggacgttctggcggaacgtcctctggtcggacgagaccaagatcgagctgttcggccacaacgaccaccggtacgtctggcgcaagaagggcgaggcctgcaagcccaagaacaccatccccacggtcaagcacggcgggggctcgatcatgctgtgggggtgcttcgcggccggcgggacgggcgccctccacaagatcgacgggatcatggacgccgtgcagtacgtggacatcctgaagcagcacctcaagacctccgtgcggaagctgaagctcggcaggaagtgggtgttccagcacgacaacgacccgaagcacacgtcgaaggtcgtggcgaagtggctgaaggacaacaaggtgaaggtgctcgagtggccctcccagtcccccgacctgaaccccatcgagaacctgtgggccgagctcaagaagcgggtgcgggcccggaggcccaccaacctcacgcagctgcaccagctctgccaggaggagtgggccaagatccaccccaactactgcggcaagctggtcgagggctacccgaagcggctcacgcaggtcaagcagttcaagggcaacgccacgaaatactgagctcgctttcttgctgtccaatttctattaaaggttcctttgttccctaagtccaactactaaactgggggatattatgaagggccttgagcatctggattctgcctaataaaaaacatttattttcattgcaagctcgctttcttgctgtccaatttctattaaaggttcctttgttccctaagtccaactactaaactgggggatattatgaagggccttgagcatctggattctgcctaataaaaaacatttattttcattgcaaaaaaaaaaaaaaaaaaaaaaaaaaaaaaaaaaaaaaaaaaaaaaaaaaaaaaaaaaaaaaaaaaaaaaaaaaaaaaaaaaaaaaaaaaaa

SEQ ID NO: 26 - RNA, 1530 nt, synthetic construct
  source 1..1530: mol_type = other RNA
acatttgcttctgacacaactgtgttcactagcaacctcaaacagacaccatgctcgctcttaagctggcgggactggacatccaatatttcaagtccaagctgggcggaggtgccccagctgttggaggtggcccgaaggctgccgacaagggtaagtccaaggagatctcgcaggacctccgcaagcggatcgtggacctccacaagtccggcagctccctcggggccatctccaagcgcctggccgtcccgcggtcgtccgtgcagacgatcgtccggaagtacaagcaccacggcaccacgcagccgtcgtacaggtcgggccgccgccgggtgctcagcccccgggacgagcggacgctcgtccggaaggtccagatcaacccgcggaccaccgcgaaggacctcgtcaagatgctcgaggagacgggcaccaaggtgtcgatctccacggtgaagcgggtcctctaccggcacaacctcaaggggcactccgcgcggaagaagcccctgctccagaaccgccacaagaaggcccgcctgcgcttcgccaccgcccacggggacaaggaccggacgttctggcggaacgtcctctggtcggacgagaccaagatcgagctgttcggccacaacgaccaccggtacgtctggcgcaagaagggcgaggcctgcaagcccaagaacaccatccccacggtcaagcacggcgggggctcgatcatgctgtgggggtgcttcgcggccggcgggacgggcgccctccacaagatcgacgggatcatggacgccgtgcagtacgtggacatcctgaagcagcacctcaagacctccgtgcggaagctgaagctcggcaggaagtgggtgttccagcacgacaacgacccgaagcacacgtcgaaggtcgtggcgaagtggctgaaggacaacaaggtgaaggtgctcgagtggccctcccagtcccccgacctgaaccccatcgagaacctgtgggccgagctcaagaagcgggtgcgggcccggaggcccaccaacctcacgcagctgcaccagctctgccaggaggagtgggccaagatccaccccaactactgcggcaagctggtcgagggctacccgaagcggctcacgcaggtcaagcagttcaagggcaacgccacgaaatactgagctcgctttcttgctgtccaatttctattaaaggttcctttgttccctaagtccaactactaaactgggggatattatgaagggccttgagcatctggattctgcctaataaaaaacatttattttcattgcaagctcgctttcttgctgtccaatttctattaaaggttcctttgttccctaagtccaactactaaactgggggatattatgaagggccttgagcatctggattctgcctaataaaaaacatttattttcattgcaaaaaaaaaaaaaaaaaaaaaaaaaaaaaaaaaaaaaaaaaaaaaaaaaaaaaaaaaaaaaaaaaaaaaaaaaaaaaaaaaaaaaaaaaaaa

SEQ ID NO: 27 - RNA, 1530 nt, synthetic construct
  source 1..1530: mol_type = other RNA
acatttgcttctgacacaactgtgttcactagcaacctcaaacagacaccatgctcgctcttaagctggcgggactggacatcctcaagtccttccaaaagctgggcggaggtgccccagctgttggaggtggcccgaaggctgccgacaagggtaagtccaaggagatctcgcaggacctccgcaagcggatcgtggacctccacaagtccggcagctccctcggggccatctccaagcgcctggccgtcccgcggtcgtccgtgcagacgatcgtccggaagtacaagcaccacggcaccacgcagccgtcgtacaggtcgggccgccgccgggtgctcagcccccgggacgagcggacgctcgtccggaaggtccagatcaacccgcggaccaccgcgaaggacctcgtcaagatgctcgaggagacgggcaccaaggtgtcgatctccacggtgaagcgggtcctctaccggcacaacctcaaggggcactccgcgcggaagaagcccctgctccagaaccgccacaagaaggcccgcctgcgcttcgccaccgcccacggggacaaggaccggacgttctggcggaacgtcctctggtcggacgagaccaagatcgagctgttcggccacaacgaccaccggtacgtctggcgcaagaagggcgaggcctgcaagcccaagaacaccatccccacggtcaagcacggcgggggctcgatcatgctgtgggggtgcttcgcggccggcgggacgggcgccctccacaagatcgacgggatcatggacgccgtgcagtacgtggacatcctgaagcagcacctcaagacctccgtgcggaagctgaagctcggcaggaagtgggtgttccagcacgacaacgacccgaagcacacgtcgaaggtcgtggcgaagtggctgaaggacaacaaggtgaaggtgctcgagtggccctcccagtcccccgacctgaaccccatcgagaacctgtgggccgagctcaagaagcgggtgcgggcccggaggcccaccaacctcacgcagctgcaccagctctgccaggaggagtgggccaagatccaccccaactactgcggcaagctggtcgagggctacccgaagcggctcacgcaggtcaagcagttcaagggcaacgccacgaaatactgagctcgctttcttgctgtccaatttctattaaaggttcctttgttccctaagtccaactactaaactgggggatattatgaagggccttgagcatctggattctgcctaataaaaaacatttattttcattgcaagctcgctttcttgctgtccaatttctattaaaggttcctttgttccctaagtccaactactaaactgggggatattatgaagggccttgagcatctggattctgcctaataaaaaacatttattttcattgcaaaaaaaaaaaaaaaaaaaaaaaaaaaaaaaaaaaaaaaaaaaaaaaaaaaaaaaaaaaaaaaaaaaaaaaaaaaaaaaaaaaaaaaaaaaa

SEQ ID NO: 28 - RNA, 1530 nt, synthetic construct
  source 1..1530: mol_type = other RNA
acatttgcttctgacacaactgtgttcactagcaacctcaaacagacaccatgctcgctcttaagctggcgggactggacatcctcaagaccttccaaaagctgggcggaggtgccccagctgttggaggtggcccgaaggctgccgacaagggtaagtccaaggagatctcgcaggacctccgcaagcggatcgtggacctccacaagtccggcagctccctcggggccatctccaagcgcctggccgtcccgcggtcgtccgtgcagacgatcgtccggaagtacaagcaccacggcaccacgcagccgtcgtacaggtcgggccgccgccgggtgctcagcccccgggacgagcggacgctcgtccggaaggtccagatcaacccgcggaccaccgcgaaggacctcgtcaagatgctcgaggagacgggcaccaaggtgtcgatctccacggtgaagcgggtcctctaccggcacaacctcaaggggcactccgcgcggaagaagcccctgctccagaaccgccacaagaaggcccgcctgcgcttcgccaccgcccacggggacaaggaccggacgttctggcggaacgtcctctggtcggacgagaccaagatcgagctgttcggccacaacgaccaccggtacgtctggcgcaagaagggcgaggcctgcaagcccaagaacaccatccccacggtcaagcacggcgggggctcgatcatgctgtgggggtgcttcgcggccggcgggacgggcgccctccacaagatcgacgggatcatggacgccgtgcagtacgtggacatcctgaagcagcacctcaagacctccgtgcggaagctgaagctcggcaggaagtgggtgttccagcacgacaacgacccgaagcacacgtcgaaggtcgtggcgaagtggctgaaggacaacaaggtgaaggtgctcgagtggccctcccagtcccccgacctgaaccccatcgagaacctgtgggccgagctcaagaagcgggtgcgggcccggaggcccaccaacctcacgcagctgcaccagctctgccaggaggagtgggccaagatccaccccaactactgcggcaagctggtcgagggctacccgaagcggctcacgcaggtcaagcagttcaagggcaacgccacgaaatactgagctcgctttcttgctgtccaatttctattaaaggttcctttgttccctaagtccaactactaaactgggggatattatgaagggccttgagcatctggattctgcctaataaaaaacatttattttcattgcaagctcgctttcttgctgtccaatttctattaaaggttcctttgttccctaagtccaactactaaactgggggatattatgaagggccttgagcatctggattctgcctaataaaaaacatttattttcattgcaaaaaaaaaaaaaaaaaaaaaaaaaaaaaaaaaaaaaaaaaaaaaaaaaaaaaaaaaaaaaaaaaaaaaaaaaaaaaaaaaaaaaaaaaaaa

SEQ ID NO: 29 - RNA, 1530 nt, synthetic construct
  source 1..1530: mol_type = other RNA
acatttgcttctgacacaactgtgttcactagcaacctcaaacagacaccatgctcgctcttaagctggcgggactggacatcgagaagttcctccaaaagctgggcggaggtgccccagctgttggaggtggcccgaaggctgccgacaagggtaagtccaaggagatctcgcaggacctccgcaagcggatcgtggacctccacaagtccggcagctccctcggggccatctccaagcgcctggccgtcccgcggtcgtccgtgcagacgatcgtccggaagtacaagcaccacggcaccacgcagccgtcgtacaggtcgggccgccgccgggtgctcagcccccgggacgagcggacgctcgtccggaaggtccagatcaacccgcggaccaccgcgaaggacctcgtcaagatgctcgaggagacgggcaccaaggtgtcgatctccacggtgaagcgggtcctctaccggcacaacctcaaggggcactccgcgcggaagaagcccctgctccagaaccgccacaagaaggcccgcctgcgcttcgccaccgcccacggggacaaggaccggacgttctggcggaacgtcctctggtcggacgagaccaagatcgagctgttcggccacaacgaccaccggtacgtctggcgcaagaagggcgaggcctgcaagcccaagaacaccatccccacggtcaagcacggcgggggctcgatcatgctgtgggggtgcttcgcggccggcgggacgggcgccctccacaagatcgacgggatcatggacgccgtgcagtacgtggacatcctgaagcagcacctcaagacctccgtgcggaagctgaagctcggcaggaagtgggtgttccagcacgacaacgacccgaagcacacgtcgaaggtcgtggcgaagtggctgaaggacaacaaggtgaaggtgctcgagtggccctcccagtcccccgacctgaaccccatcgagaacctgtgggccgagctcaagaagcgggtgcgggcccggaggcccaccaacctcacgcagctgcaccagctctgccaggaggagtgggccaagatccaccccaactactgcggcaagctggtcgagggctacccgaagcggctcacgcaggtcaagcagttcaagggcaacgccacgaaatactgagctcgctttcttgctgtccaatttctattaaaggttcctttgttccctaagtccaactactaaactgggggatattatgaagggccttgagcatctggattctgcctaataaaaaacatttattttcattgcaagctcgctttcttgctgtccaatttctattaaaggttcctttgttccctaagtccaactactaaactgggggatattatgaagggccttgagcatctggattctgcctaataaaaaacatttattttcattgcaaaaaaaaaaaaaaaaaaaaaaaaaaaaaaaaaaaaaaaaaaaaaaaaaaaaaaaaaaaaaaaaaaaaaaaaaaaaaaaaaaaaaaaaaaaa

SEQ ID NO: 30 - protein, 10 aa, synthetic construct
LALKLAGLDI

SEQ ID NO: 31 - protein, 5 aa, synthetic construct
KFERQ

SEQ ID NO: 32 - protein, 5 aa, synthetic construct
KFSRK

SEQ ID NO: 33 - protein, 5 aa, synthetic construct
VKKDQ

SEQ ID NO: 34 - protein, 5 aa, synthetic construct
KFFEQ

SEQ ID NO: 35 - protein, 5 aa, synthetic construct
KIREI

SEQ ID NO: 36 - protein, 5 aa, synthetic construct
QVELR

SEQ ID NO: 37 - protein, 5 aa, synthetic construct
QYFKS

SEQ ID NO: 38 - protein, 5 aa, synthetic construct
LKSFQ

SEQ ID NO: 39 - protein, 5 aa, synthetic construct
LKYFQ

SEQ ID NO: 40 - protein, 5 aa, synthetic construct
EKFLQ

SEQ ID NO: 41 - protein, 5 aa, synthetic construct
QREFK

SEQ ID NO: 42 - protein, 5 aa, synthetic construct
VDKFQ

SEQ ID NO: 43 - protein, 340 aa, synthetic construct
MGKSKEISQDLRKRIVDLHKSGSSLGAISKRLAVPRSSVQTIVRKYKHHGTTQPSYRSGRRRVLSPRDERTLVRKVQINPRTTAKDLVKMLEETGTKVSISTVKRVLYRHNLKGHSARKKPLLQNRHKKARLRFATAHGDKDRTFWRNVLWSDETKIELFGHNDHRYVWRKKGEACKPKNTIPTVKHGGGSIMLWGCFAAGGTGALHKIDGIMDAVQYVDILKQHLKTSVRKLKLGRKWVFQHDNDPKHTSKVVAKWLKDNKVKVLEWPSQSPDLNPIENLWAELKKRVRARRPTNLTQLHQLCQEEWAKIHPNYCGKLVEGYPKRLTQVKQFKGNATKY

SEQ ID NO: 44 - protein, 340 aa, synthetic construct
MPRPKEIQEQLRKKVIEIYQSGKGYKAISKALGIQRTTVRAIIHKWRRHGTVVNLPRSGRPPKITPRAQRRLIQEVTKDPTTTSKELQASLASVKVSVHASTIRKRLGKNGLHGRVPRRKPLLSKKNIKARLNFSTTHLDDPQDFWDNILWTDETKVELFGRCVSKYIWRRRNTAFHKKNIIPTVKYGGGSVMVWGCFAASGPGRLAVIKGTMNSAVYQEILKENVRPSVRVLKLKRTWVLQQDNDPKHTSKSTTEWLKKNKMKTLEWPSQSPDLNPIEMLWYDLKKAVHARKPSNVTELGQFCKDEWAKIPPGRCKSLIARYRKRLVAVVAAKGGPTSY

SEQ ID NO: 45 - protein, 341 aa, Drosophila hydei
MVRGKPISKEIRVLIRDYFKSGKTLTEISKQLNLPKSSVHGVIQIFKKNGNIENNIANRGRTSAITPRDKRQLAKIVKADRRQSLRNLASKWSQTIGKTVKREWTRQQLKSIGYGFYKAKEKPLLTLRQKKKRLQWARERMSWTQRQWDTIIFSDEAKFDVSVGDTRKRVIRKRSETYHKDCLKRTTKFPASTMVWGCMSAKGLGKLHFIEGTVNAEKYINILQDSLLPSIPKLSDCGEFTFQQDGASSHTAKRTKNWLQYNQMEVLDWPSNSPDLSPIENIWWLMKNQLRNEPQRNISDLKIKLQEMWDSISQEHCKNLLSSMPKRVKCVMQAKGDVTQF

SEQ ID NO: 46 - protein, 340 aa, Danio rerio
MGKNKELSQDLRSLIVEKHFDGNGYRRISRMLNVPVSTVGAIIRKWKKHKFTINRPRSGAPRKIPVRGVQRIIRRVLQEPRTTRAELQEDLASAGTIVSKKTISNALNHHGIHARSPRKTPLLNKKHVEARLKFAKQHLEKPVDYWETIVWSDESKIELFGSHSTHHVWRRNGTAHHPKNTIPTVKFGGGSIMVWGCFSARGTGRLHIIEGRMNGEMYRDILDKNLLPSTRKLKMKRGWTFQQDNDPKHKAKETMKWFQRKKIKLLEWPSQSPDLNPIENLWRELKIKVHKRGPRNLQDLKTVCVEEWARITPEQCRRLVSPYKRRLEAVITNKGFSTKY

SEQ ID NO: 47 - protein, 339 aa, Danio rerio
MGKSKEISQDIRKRIVDLHKSGSSLVTISRCLKVPHSSVQTNLRNYKQHGNVQPSYRSGRRRILCPRDERAMVRTVCINPRTKAKDLVKMLAEAGKRVSLSTVKRVLYHGLKGHSARKKPLLQKHHKKARLQFAKLHWEKDLCFWRHVLWSDGAKIELFGHNDQRYIWRTKGKAYKPKNTIPTVQYGGGSIMLWGCFAAGGTGPLHSIDGIMRKEHYVEILKQHLKTSARKLKLGHKWVFQMDHDPKHTAKLVKMCFKDNRVNVLEWPSQSPDLNPIENLWAELKKLVRARQPTNLTQLHQFCQEEWAKIPANYCEKLVEGYPKHLTKVIQFKSKAYKY

SEQ ID NO: 48 - protein, 338 aa, Pleuronectes platessa
MKTKELTKQVRDKVVEKYEAGLGYKKISRALNISLSTIKSIIRKWKEYGTTANLPRGGRPPKLKSRTRRKLIREATRRPMVTLEELQRSTAEVGESVHRTTISRLLHKSGLYGRVARRKPLLKGIHKKSRLEFARSHVGDTANMWKKVLWSDETKIELFGLNAKRYVWRKPNTAHHPEHTIPTVKHGGGSIMLWGCFSSAGTGKLVRIEGKMDGAKYREILEENLMQSAKDLRLGRRFIFQQDNDPKHTARATKEWFGLKNVNVLKWPSQSPDLNPIENLWQDLKIAVHRRSPNLTELHLFCQEEWTNLSISRCAKLVETYPKRLAAVIAAKGGSTKY

SEQ ID NO: 49 - protein, 18 aa, synthetic construct
KLGGGAPAVGGGPKAADK

SEQ ID NO: 50 - protein, 373 aa, synthetic construct
MLALKLAGLDIKFERQKLGGGAPAVGGGPKAADKGKSKEISQDLRKRIVDLHKSGSSLGAISKRLAVPRSSVQTIVRKYKHHGTTQPSYRSGRRRVLSPRDERTLVRKVQINPRTTAKDLVKMLEETGTKVSISTVKRVLYRHNLKGHSARKKPLLQNRHKKARLRFATAHGDKDRTFWRNVLWSDETKIELFGHNDHRYVWRKKGEACKPKNTIPTVKHGGGSIMLWGCFAAGGTGALHKIDGIMDAVQYVDILKQHLKTSVRKLKLGRKWVFQHDNDPKHTSKVVAKWLKDNKVKVLEWPSQSPDLNPIENLWAELKKRVRARRPTNLTQLHQLCQEEWAKIHPNYCGKLVEGYPKRLTQVKQFKGNATKY

SEQ ID NO: 51 - RNA, 50 nt, Homo sapiens
  source 1..50: mol_type = mRNA
acatttgcttctgacacaactgtgttcactagcaacctcaaacagacacc

SEQ ID NO: 52 - RNA, 45 nt, synthetic construct
  source 1..45: mol_type = other RNA
actcactatttgttttcgcgcccagttgcaaaaagtgtcgccacc

SEQ ID NO: 53 - RNA, 134 nt, Homo sapiens
  source 1..134: mol_type = mRNA
gctcgctttcttgctgtccaatttctattaaaggttcctttgttccctaagtccaactactaaactgggggatattatgaagggccttgagcatctggattctgcctaataaaaaacatttattttcattgcaa

SEQ ID NO: 54 - RNA, 110 nt, Homo sapiens
  source 1..110: mol_type = mRNA
gctggagcctcggtagccgttcctcctgcccgctgggcctcccaacgggccctcctcccctccttgcaccggcccttcctggtctttgaataaagtctgagtgggcagca

SEQ ID NO: 55 - RNA, 589 nt, synthetic construct
  source 1..589: mol_type = other RNA
aatcaacctctggattacaaaatttgtgaaagattgactggtattcttaactatgttgctccttttacgctatgtggatacgctgctttaatgcctttgtatcatgctattgcttcccgtatggctttcattttctcctccttgtataaatcctggttgctgtctctttatgaggagttgtggcccgttgtcaggcaacgtggcgtggtgtgcactgtgtttgctgacgcaacccccactggttggggcattgccaccacctgtcagctcctttccgggactttcgctttccccctccctattgccacggcggaactcatcgccgcctgccttgcccgctgctggacaggggctcggctgttgggcactgacaattccgtggtgttgtcggggaagctgacgtcctttccatggctgctcgcctgtgttgccacctggattctgcgcgggacgtccttctgctacgtcccttcggccctcaatccagcggaccttccttcccgcggcctgctgccggctctgcggcctcttccgcgtcttggccttcgccctcagacgagtcggatctccctttgggccgcctccccgc

SEQ ID NO: 56 - RNA, 244 nt, synthetic construct
  source 1..244: mol_type = other RNA
gctcgctttcttgctgtccaatttctattaaaggttcctttgttccctaagtccaactactaaactgggggatattatgaagggccttgagcatctggattctgcctaataaaaaacatttattttcattgcaagctggagcctcggtagccgttcctcctgcccgctgggcctcccaacgggccctcctcccctccttgcaccggcccttcctggtctttgaataaagtctgagtgggcagca

SEQ ID NO: 57 - RNA, 107 nt, synthetic construct
  source 1..107: mol_type = other RNA
gctcgctttcttgctgtccaatttctattaaaggttcctttgttccctaagtccaactactaaactgggggatattatgaagggccttgagcatctggattctgcct

SEQ ID NO: 58 - RNA, 1023 nt, synthetic construct
  source 1..1023: mol_type = other RNA
atgggcaaatccaaggagatctcccaggacctgaggaaaagaatcgtggacctgcacaaatctggctcttctctgggcgccatctctaaaagactggccgtgcctaggtccagcgtgcagaccattgtgcggaaatacaaacaccacggaaccacacagccatcttaccgctccggacggcggagagtgctgtcccctagagacgagaggaccctcgtgagaaaagtgcagatcaaccctagaacaaccgccaaagacctggtgaaaatgctggaggagaccggcaccaaggtgtccatctctaccgtgaagcgcgtgctgtaccggcacaacctgaagggacactccgcccggaagaaacctctgctgcagaataggcacaagaaagcccggctgagattcgccaccgcccacggcgataaggatagaaccttttggcgcaacgtgctgtggagcgacgagacaaaaatcgagctgttcgggcacaacgatcaccgctacgtgtggcgcaaaaagggagaggcctgtaagccaaaaaacaccatccccaccgtgaaacacggcggaggctccattatgctgtggggctgctttgccgccggcggaaccggagccctgcacaaaatcgacggcatcatggatgccgtgcagtacgtggacatcctgaaacagcacctgaaaacctctgtgagaaaactgaaactgggccgcaaatgggtgttccagcacgacaatgaccctaagcacacatccaaagtggtggccaaatggctgaaagacaacaaagtgaaagtgctggagtggccttcccagtcccccgatctgaacccaattgagaacctgtgggccgagctgaagaaaagagtgcgggccagacggcctacaaacctgacacagctgcaccagctgtgtcaggaggagtgggccaaaatccaccccaactactgtggcaagctggtggagggatacccaaaacggctgacccaagtgaaacagttcaagggcaacgccaccaagtactga

SEQ ID NO: 59 - RNA, 1122 nt, synthetic construct
  source 1..1122: mol_type = other RNA
atgctggctctgaaactggccggcctggacatcaagttcgagagacagaaactcggcggaggcgcccctgctgttggcggaggacctaaagctgctgacaagggcaaatccaaggagatctcccaggacctgaggaaaagaatcgtggacctgcacaaatctggctcttctctgggcgccatctctaaaagactggccgtgcctaggtccagcgtgcagaccattgtgcggaaatacaaacaccacggaaccacacagccatcttaccgctccggacggcggagagtgctgtcccctagagacgagaggaccctcgtgagaaaagtgcagatcaaccctagaacaaccgccaaagacctggtgaaaatgctggaggagaccggcaccaaggtgtccatctctaccgtgaagcgcgtgctgtaccggcacaacctgaagggacactccgcccggaagaaacctctgctgcagaataggcacaagaaagcccggctgagattcgccaccgcccacggcgataaggatagaaccttttggcgcaacgtgctgtggagcgacgagacaaaaatcgagctgttcgggcacaacgatcaccgctacgtgtggcgcaaaaagggagaggcctgtaagccaaaaaacaccatccccaccgtgaaacacggcggaggctccattatgctgtggggctgctttgccgccggcggaaccggagccctgcacaaaatcgacggcatcatggatgccgtgcagtacgtggacatcctgaaacagcacctgaaaacctctgtgagaaaactgaaactgggccgcaaatgggtgttccagcacgacaatgaccctaagcacacatccaaagtggtggccaaatggctgaaagacaacaaagtgaaagtgctggagtggccttcccagtcccccgatctgaacccaattgagaacctgtgggccgagctgaagaaaagagtgcgggccagacggcctacaaacctgacacagctgcaccagctgtgtcaggaggagtgggccaaaatccaccccaactactgtggcaagctggtggagggatacccaaaacggctgacccaagtgaaacagttcaagggcaacgccaccaagtactga

SEQ ID NO: 60 - protein, 15 aa, synthetic construct
LALKLAGLDIKFERQ

SEQ ID NO: 61 - RNA, 67 nt, synthetic construct
  source 1..67: mol_type = other RNA
ataattcaaaatcaatcagcatcacaacatcaagcatcaatcatcaacacatcaaagagacaccacc

SEQ ID NO: 62 - RNA, 1761 nt, synthetic construct
  source 1..1761: mol_type = other RNA
acatttgcttctgacacaactgtgttcactagcaacctcaaacagacaccatgctggctctgaaactggccggcctggacatcaagttcgagagacagaaactcggcggaggcgcccctgctgttggcggaggacctaaagctgctgacaagggcaaatccaaggagatctcccaggacctgaggaaaagaatcgtggacctgcacaaatctggctcttctctgggcgccatctctaaaagactggccgtgcctaggtccagcgtgcagaccattgtgcggaaatacaaacaccacggaaccacacagccatcttaccgctccggacggcggagagtgctgtcccctagagacgagaggaccctcgtgagaaaagtgcagatcaaccctagaacaaccgccaaagacctggtgaaaatgctggaggagaccggcaccaaggtgtccatctctaccgtgaagcgcgtgctgtaccggcacaacctgaagggacactccgcccggaagaaacctctgctgcagaataggcacaagaaagcccggctgagattcgccaccgcccacggcgataaggatagaaccttttggcgcaacgtgctgtggagcgacgagacaaaaatcgagctgttcgggcacaacgatcaccgctacgtgtggcgcaaaaagggagaggcctgtaagccaaaaaacaccatccccaccgtgaaacacggcggaggctccattatgctgtggggctgctttgccgccggcggaaccggagccctgcacaaaatcgacggcatcatggatgccgtgcagtacgtggacatcctgaaacagcacctgaaaacctctgtgagaaaactgaaactgggccgcaaatgggtgttccagcacgacaatgaccctaagcacacatccaaagtggtggccaaatggctgaaagacaacaaagtgaaagtgctggagtggccttcccagtcccccgatctgaacccaattgagaacctgtgggccgagctgaagaaaagagtgcgggccagacggcctacaaacctgacacagctgcaccagctgtgtcaggaggagtgggccaaaatccaccccaactactgtggcaagctggtggagggatacccaaaacggctgacccaagtgaaacagttcaagggcaacgccaccaagtactgaaatcaacctctggattacaaaatttgtgaaagattgactggtattcttaactatgttgctccttttacgctatgtggatacgctgctttaatgcctttgtatcatgctattgcttcccgtatggctttcattttctcctccttgtataaatcctggttgctgtctctttatgaggagttgtggcccgttgtcaggcaacgtggcgtggtgtgcactgtgtttgctgacgcaacccccactggttggggcattgccaccacctgtcagctcctttccgggactttcgctttccccctccctattgccacggcggaactcatcgccgcctgccttgcccgctgctggacaggggctcggctgttgggcactgacaattccgtggtgttgtcggggaagctgacgtcctttccatggctgctcgcctgtgttgccacctggattctgcgcgggacgtccttctgctacgtcccttcggccctcaatccagcggaccttccttcccgcggcctgctgccggctctgcggcctcttccgcgtcttggccttcgccctcagacgagtcggatctccctttgggccgcctccccgc

SEQ ID NO: 63 - RNA, 1306 nt, synthetic construct
  source 1..1306: mol_type = other RNA
acatttgcttctgacacaactgtgttcactagcaacctcaaacagacaccatgctggctctgaaactggccggcctggacatcaagttcgagagacagaaactcggcggaggcgcccctgctgttggcggaggacctaaagctgctgacaagggcaaatccaaggagatctcccaggacctgaggaaaagaatcgtggacctgcacaaatctggctcttctctgggcgccatctctaaaagactggccgtgcctaggtccagcgtgcagaccattgtgcggaaatacaaacaccacggaaccacacagccatcttaccgctccggacggcggagagtgctgtcccctagagacgagaggaccctcgtgagaaaagtgcagatcaaccctagaacaaccgccaaagacctggtgaaaatgctggaggagaccggcaccaaggtgtccatctctaccgtgaagcgcgtgctgtaccggcacaacctgaagggacactccgcccggaagaaacctctgctgcagaataggcacaagaaagcccggctgagattcgccaccgcccacggcgataaggatagaaccttttggcgcaacgtgctgtggagcgacgagacaaaaatcgagctgttcgggcacaacgatcaccgctacgtgtggcgcaaaaagggagaggcctgtaagccaaaaaacaccatccccaccgtgaaacacggcggaggctccattatgctgtggggctgctttgccgccggcggaaccggagccctgcacaaaatcgacggcatcatggatgccgtgcagtacgtggacatcctgaaacagcacctgaaaacctctgtgagaaaactgaaactgggccgcaaatgggtgttccagcacgacaatgaccctaagcacacatccaaagtggtggccaaatggctgaaagacaacaaagtgaaagtgctggagtggccttcccagtcccccgatctgaacccaattgagaacctgtgggccgagctgaagaaaagagtgcgggccagacggcctacaaacctgacacagctgcaccagctgtgtcaggaggagtgggccaaaatccaccccaactactgtggcaagctggtggagggatacccaaaacggctgacccaagtgaaacagttcaagggcaacgccaccaagtactgagctcgctttcttgctgtccaatttctattaaaggttcctttgttccctaagtccaactactaaactgggggatattatgaagggccttgagcatctggattctgcctaataaaaaacatttattttcattgcaa

SEQ ID NO: 64 - RNA, 1282 nt, synthetic construct
  source 1..1282: mol_type = other RNA
acatttgcttctgacacaactgtgttcactagcaacctcaaacagacaccatgctggctctgaaactggccggcctggacatcaagttcgagagacagaaactcggcggaggcgcccctgctgttggcggaggacctaaagctgctgacaagggcaaatccaaggagatctcccaggacctgaggaaaagaatcgtggacctgcacaaatctggctcttctctgggcgccatctctaaaagactggccgtgcctaggtccagcgtgcagaccattgtgcggaaatacaaacaccacggaaccacacagccatcttaccgctccggacggcggagagtgctgtcccctagagacgagaggaccctcgtgagaaaagtgcagatcaaccctagaacaaccgccaaagacctggtgaaaatgctggaggagaccggcaccaaggtgtccatctctaccgtgaagcgcgtgctgtaccggcacaacctgaagggacactccgcccggaagaaacctctgctgcagaataggcacaagaaagcccggctgagattcgccaccgcccacggcgataaggatagaaccttttggcgcaacgtgctgtggagcgacgagacaaaaatcgagctgttcgggcacaacgatcaccgctacgtgtggcgcaaaaagggagaggcctgtaagccaaaaaacaccatccccaccgtgaaacacggcggaggctccattatgctgtggggctgctttgccgccggcggaaccggagccctgcacaaaatcgacggcatcatggatgccgtgcagtacgtggacatcctgaaacagcacctgaaaacctctgtgagaaaactgaaactgggccgcaaatgggtgttccagcacgacaatgaccctaagcacacatccaaagtggtggccaaatggctgaaagacaacaaagtgaaagtgctggagtggccttcccagtcccccgatctgaacccaattgagaacctgtgggccgagctgaagaaaagagtgcgggccagacggcctacaaacctgacacagctgcaccagctgtgtcaggaggagtgggccaaaatccaccccaactactgtggcaagctggtggagggatacccaaaacggctgacccaagtgaaacagttcaagggcaacgccaccaagtactgagctggagcctcggtagccgttcctcctgcccgctgggcctcccaacgggccctcctcccctccttgcaccggcccttcctggtctttgaataaagtctgagtgggcagca

SEQ ID NO: 65 - RNA, 1416 nt, synthetic construct
  source 1..1416: mol_type = other RNA
acatttgcttctgacacaactgtgttcactagcaacctcaaacagacaccatgctggctctgaaactggccggcctggacatcaagttcgagagacagaaactcggcggaggcgcccctgctgttggcggaggacctaaagctgctgacaagggcaaatccaaggagatctcccaggacctgaggaaaagaatcgtggacctgcacaaatctggctcttctctgggcgccatctctaaaagactggccgtgcctaggtccagcgtgcagaccattgtgcggaaatacaaacaccacggaaccacacagccatcttaccgctccggacggcggagagtgctgtcccctagagacgagaggaccctcgtgagaaaagtgcagatcaaccctagaacaaccgccaaagacctggtgaaaatgctggaggagaccggcaccaaggtgtccatctctaccgtgaagcgcgtgctgtaccggcacaacctgaagggacactccgcccggaagaaacctctgctgcagaataggcacaagaaagcccggctgagattcgccaccgcccacggcgataaggatagaaccttttggcgcaacgtgctgtggagcgacgagacaaaaatcgagctgttcgggcacaacgatcaccgctacgtgtggcgcaaaaagggagaggcctgtaagccaaaaaacaccatccccaccgtgaaacacggcggaggctccattatgctgtggggctgctttgccgccggcggaaccggagccctgcacaaaatcgacggcatcatggatgccgtgcagtacgtggacatcctgaaacagcacctgaaaacctctgtgagaaaactgaaactgggccgcaaatgggtgttccagcacgacaatgaccctaagcacacatccaaagtggtggccaaatggctgaaagacaacaaagtgaaagtgctggagtggccttcccagtcccccgatctgaacccaattgagaacctgtgggccgagctgaagaaaagagtgcgggccagacggcctacaaacctgacacagctgcaccagctgtgtcaggaggagtgggccaaaatccaccccaactactgtggcaagctggtggagggatacccaaaacggctgacccaagtgaaacagttcaagggcaacgccaccaagtactgagctcgctttcttgctgtccaatttctattaaaggttcctttgttccctaagtccaactactaaactgggggatattatgaagggccttgagcatctggattctgcctaataaaaaacatttattttcattgcaagctggagcctcggtagccgttcctcctgcccgctgggcctcccaacgggccctcctcccctccttgcaccggcccttcctggtctttgaataaagtctgagtgggcagca

SEQ ID NO: 66 - RNA, 1279 nt, synthetic construct
  source 1..1279: mol_type = other RNA
acatttgcttctgacacaactgtgttcactagcaacctcaaacagacaccatgctggctctgaaactggccggcctggacatcaagttcgagagacagaaactcggcggaggcgcccctgctgttggcggaggacctaaagctgctgacaagggcaaatccaaggagatctcccaggacctgaggaaaagaatcgtggacctgcacaaatctggctcttctctgggcgccatctctaaaagactggccgtgcctaggtccagcgtgcagaccattgtgcggaaatacaaacaccacggaaccacacagccatcttaccgctccggacggcggagagtgctgtcccctagagacgagaggaccctcgtgagaaaagtgcagatcaaccctagaacaaccgccaaagacctggtgaaaatgctggaggagaccggcaccaaggtgtccatctctaccgtgaagcgcgtgctgtaccggcacaacctgaagggacactccgcccggaagaaacctctgctgcagaataggcacaagaaagcccggctgagattcgccaccgcccacggcgataaggatagaaccttttggcgcaacgtgctgtggagcgacgagacaaaaatcgagctgttcgggcacaacgatcaccgctacgtgtggcgcaaaaagggagaggcctgtaagccaaaaaacaccatccccaccgtgaaacacggcggaggctccattatgctgtggggctgctttgccgccggcggaaccggagccctgcacaaaatcgacggcatcatggatgccgtgcagtacgtggacatcctgaaacagcacctgaaaacctctgtgagaaaactgaaactgggccgcaaatgggtgttccagcacgacaatgaccctaagcacacatccaaagtggtggccaaatggctgaaagacaacaaagtgaaagtgctggagtggccttcccagtcccccgatctgaacccaattgagaacctgtgggccgagctgaagaaaagagtgcgggccagacggcctacaaacctgacacagctgcaccagctgtgtcaggaggagtgggccaaaatccaccccaactactgtggcaagctggtggagggatacccaaaacggctgacccaagtgaaacagttcaagggcaacgccaccaagtactgagctcgctttcttgctgtccaatttctattaaaggttcctttgttccctaagtccaactactaaactgggggatattatgaagggccttgagcatctggattctgcct

SEQ ID NO: 67 - RNA, 1435 nt, synthetic construct
  source 1..1435: mol_type = other RNA
actcactatttgttttcgcgcccagttgcaaaaagtgtcgccaccatgctggctctgaaactggccggcctggacatcaagttcgagagacagaaactcggcggaggcgcccctgctgttggcggaggacctaaagctgctgacaagggcaaatccaaggagatctcccaggacctgaggaaaagaatcgtggacctgcacaaatctggctcttctctgggcgccatctctaaaagactggccgtgcctaggtccagcgtgcagaccattgtgcggaaatacaaacaccacggaaccacacagccatcttaccgctccggacggcggagagtgctgtcccctagagacgagaggaccctcgtgagaaaagtgcagatcaaccctagaacaaccgccaaagacctggtgaaaatgctggaggagaccggcaccaaggtgtccatctctaccgtgaagcgcgtgctgtaccggcacaacctgaagggacactccgcccggaagaaacctctgctgcagaataggcacaagaaagcccggctgagattcgccaccgcccacggcgataaggatagaaccttttggcgcaacgtgctgtggagcgacgagacaaaaatcgagctgttcgggcacaacgatcaccgctacgtgtggcgcaaaaagggagaggcctgtaagccaaaaaacaccatccccaccgtgaaacacggcggaggctccattatgctgtggggctgctttgccgccggcggaaccggagccctgcacaaaatcgacggcatcatggatgccgtgcagtacgtggacatcctgaaacagcacctgaaaacctctgtgagaaaactgaaactgggccgcaaatgggtgttccagcacgacaatgaccctaagcacacatccaaagtggtggccaaatggctgaaagacaacaaagtgaaagtgctggagtggccttcccagtcccccgatctgaacccaattgagaacctgtgggccgagctgaagaaaagagtgcgggccagacggcctacaaacctgacacagctgcaccagctgtgtcaggaggagtgggccaaaatccaccccaactactgtggcaagctggtggagggatacccaaaacggctgacccaagtgaaacagttcaagggcaacgccaccaagtactgagctcgctttcttgctgtccaatttctattaaaggttcctttgttccctaagtccaactactaaactgggggatattatgaagggccttgagcatctggattctgcctaataaaaaacatttattttcattgcaagctcgctttcttgctgtccaatttctattaaaggttcctttgttccctaagtccaactactaaactgggggatattatgaagggccttgagcatctggattctgcctaataaaaaacatttattttcattgcaa

SEQ ID NO: 68 - RNA, 1435 nt, synthetic construct
  source 1..1435: mol_type = other RNA
actcactatttgttttcgcgcccagttgcaaaaagtgtcgccaccatgctagcactaaaactcgcgggactcgatatcaagttcgaaagacagaagctgggcggcggcgccccggccgtgggcgggggcccgaaggccgccgacaagggcaagtccaaggagatctcgcaggacctccgcaagcggatcgtggacctccacaagtccggcagctccctcggggccatctccaagcgcctggccgtcccgcggtcgtccgtgcagacgatcgtccggaagtacaagcaccacggcaccacgcagccgtcgtacaggtcgggccgccgccgggtgctcagcccccgggacgagcggacgctcgtccggaaggtccagatcaacccgcggaccaccgcgaaggacctcgtcaagatgctcgaggagacgggcaccaaggtgtcgatctccacggtgaagcgggtcctctaccggcacaacctcaaggggcactccgcgcggaagaagcccctgctccagaaccgccacaagaaggcccgcctgcgcttcgccaccgcccacggggacaaggaccggacgttctggcggaacgtcctctggtcggacgagaccaagatcgagctgttcggccacaacgaccaccggtacgtctggcgcaagaagggcgaggcctgcaagcccaagaacaccatccccacggtcaagcacggcgggggctcgatcatgctgtgggggtgcttcgcggccggcgggacgggcgccctccacaagatcgacgggatcatggacgccgtgcagtacgtggacatcctgaagcagcacctcaagacctccgtgcggaagctgaagctcggcaggaagtgggtgttccagcacgacaacgacccgaagcacacgtcgaaggtcgtggcgaagtggctgaaggacaacaaggtgaaggtgctcgagtggccctcccagtcccccgacctgaaccccatcgagaacctgtgggccgagctcaagaagcgggtgcgggcccggaggcccaccaacctcacgcagctgcaccagctctgccaggaggagtgggccaagatccaccccaactactgcggcaagctggtcgagggctacccgaagcggctcacgcaggtcaagcagttcaagggcaacgccacgaaatactgagctcgctttcttgctgtccaatttctattaaaggttcctttgttccctaagtccaactactaaactgggggatattatgaagggccttgagcatctggattctgcctaataaaaaacatttattttcattgcaagctcgctttcttgctgtccaatttctattaaaggttcctttgttccctaagtccaactactaaactgggggatattatgaagggccttgagcatctggattctgcctaataaaaaacatttattttcattgcaa

SEQ ID NO: 69 - RNA, 1440 nt, synthetic construct
  source 1..1440: mol_type = other RNA
acatttgcttctgacacaactgtgttcactagcaacctcaaacagacaccatgctcgccctcaagctggcggggctggacatcaagttcgagcgccagaagctgggcggcggcgccccggccgtgggcgggggcccgaaggccgccgacaagggcaagtccaaggagatctcgcaggacctccgcaagcggatcgtggacctccacaagtccggcagctccctcggggccatctccaagcgcctggccgtcccgcggtcgtccgtgcagacgatcgtccggaagtacaagcaccacggcaccacgcagccgtcgtacaggtcgggccgccgccgggtgctcagcccccgggacgagcggacgctcgtccggaaggtccagatcaacccgcggaccaccgcgaaggacctcgtcaagatgctcgaggagacgggcaccaaggtgtcgatctccacggtgaagcgggtcctctaccggcacaacctcaaggggcactccgcgcggaagaagcccctgctccagaaccgccacaagaaggcccgcctgcgcttcgccaccgcccacggggacaaggaccggacgttctggcggaacgtcctctggtcggacgagaccaagatcgagctgttcggccacaacgaccaccggtacgtctggcgcaagaagggcgaggcctgcaagcccaagaacaccatccccacggtcaagcacggcgggggctcgatcatgctgtgggggtgcttcgcggccggcgggacgggcgccctccacaagatcgacgggatcatggacgccgtgcagtacgtggacatcctgaagcagcacctcaagacctccgtgcggaagctgaagctcggcaggaagtgggtgttccagcacgacaacgacccgaagcacacgtcgaaggtcgtggcgaagtggctgaaggacaacaaggtgaaggtgctcgagtggccctcccagtcccccgacctgaaccccatcgagaacctgtgggccgagctcaagaagcgggtgcgggcccggaggcccaccaacctcacgcagctgcaccagctctgccaggaggagtgggccaagatccaccccaactactgcggcaagctggtcgagggctacccgaagcggctcacgcaggtcaagcagttcaagggcaacgccacgaaatactgagctcgctttcttgctgtccaatttctattaaaggttcctttgttccctaagtccaactactaaactgggggatattatgaagggccttgagcatctggattctgcctaataaaaaacatttattttcattgcaagctcgctttcttgctgtccaatttctattaaaggttcctttgttccctaagtccaactactaaactgggggatattatgaagggccttgagcatctggattctgcctaataaaaaacatttattttcattgcaa